European Patent Application EP 4 130 283 A1, published February 8, 2023. Title: Nucleic acid construct capable of measuring homologous recombination activity and use of the same. Applicant: Public University Corporation Yokohama City University. The sequence listing filed with the application follows.

SEQUENCE LISTING (48 sequences)

SEQ ID NO: 1 - DNA, 45 bp, Artificial Sequence
  primer DTA-Fw
actcactataggctagcgtcctcgccatggatcctgatgatgttg

SEQ ID NO: 2 - DNA, 40 bp, Artificial Sequence
  primer Sce-5'DTA-Rv
attaccctgttatccctatcattgtgtaccagattttggc

SEQ ID NO: 3 - DNA, 41 bp, Artificial Sequence
  primer Sce-3'DTA-Fw
tagggataacagggtaataaagggttttatagtaccgacaa

SEQ ID NO: 4 - DNA, 46 bp, Artificial Sequence
  primer DTA-Rv
ccgccccgactctagaatcacaaagatcgcctgacacgatttcctg

SEQ ID NO: 5 - DNA, 42 bp, Artificial Sequence
  primer iDTA-Fw
aaatgtggtaaaatcgatgaattacagctcttaaggctagag

SEQ ID NO: 6 - DNA, 42 bp, Artificial Sequence
  primer iDTA-Rv
acgcggatccttatcgtcagacttgctccatcaacggttcag

SEQ ID NO: 7 - DNA, 23 bp, Artificial Sequence
  primer Nluc-Fw
taatacgactcactataggctag

SEQ ID NO: 8 - DNA, 43 bp, Artificial Sequence
  primer Sce-5'Nluc-Rv
attaccctgttatccctatcactggcccatttggtcgccgctc

SEQ ID NO: 9 - DNA, 45 bp, Artificial Sequence
  primer Sce-3'Nluc-Fw
tgatagggataacagggtaatgtgtaccctgtggatgatcatcac

SEQ ID NO: 10 - DNA, 23 bp, Artificial Sequence
  primer Nluc-Rv
ccgccccgactctagagtcgcgg

SEQ ID NO: 11 - DNA, 44 bp, Artificial Sequence
  primer iNluc-Fw
aaatcgataaggatcgctagcatgaagatttcgttggggactgg

SEQ ID NO: 12 - DNA, 44 bp, Artificial Sequence
  primer iNluc-Rv
caccatacgcggatccttatcagttgatggttactcggaacagc

SEQ ID NO: 13 - DNA, 591 bp, Corynebacterium diphtheriae
  CDS (1)..(591)
atggatcctgatgatgttgttgattcttctaaatcttttgtgatggaaaacttttcttcgtaccacgggactaaacctggttatgtagattccattcaaaaaggtatacaaaagccaaaatctggtacacaaggaaattatgacgatgattggaaagggttttatagtaccgacaataaatacgacgctgcgggatactctgtagataatgaaaacccgctctctggaaaagctggaggcgtggtcaaagtgacgtatccaggactgacgaaggttctcgcactaaaagtggataatgccgaaactattaagaaagagttaggtttaagtctcactgaaccgttgatggagcaagtcggaacggaagagtttatcaaaaggttcggtgatggtgcttcgcgtgtagtgctcagccttcccttcgctgaggggagttctagcgttgaatatattaataactgggaacaggcgaaagcgttaagcgtagaacttgagattaattttgaaacccgtggaaaacgtggccaagatgcgatgtatgagtatatggctcaagcctgtgcaggaaatcgtgtcaggcgatctttgtga

SEQ ID NO: 14 - protein, 196 aa, Corynebacterium diphtheriae
MDPDDVVDSSKSFVMENFSSYHGTKPGYVDSIQKGIQKPKSGTQGNYDDDWKGFYSTDNKYDAAGYSVDNENPLSGKAGGVVKVTYPGLTKVLALKVDNAETIKKELGLSLTEPLMEQVGTEEFIKRFGDGASRVVLSLPFAEGSSSVEYINNWEQAKALSVELEINFETRGKRGQDAMYEYMAQACAGNRVRRSL

SEQ ID NO: 15 - DNA, 588 bp, Artificial Sequence
  SceDTA fragment
  CDS (1)..(588)
atggatcctgatgatgttgttgattcttctaaatcttttgtgatggaaaacttttcttcgtaccacgggactaaacctggttatgtagattccattcaaaaaggtatacaaaagccaaaatctggtacacaatgatagggataacagggtaataaagggttttatagtaccgacaataaatacgacgctgcgggatactctgtagataatgaaaacccgctctctggaaaagctggaggcgtggtcaaagtgacgtatccaggactgacgaaggttctcgcactaaaagtggataatgccgaaactattaagaaagagttaggtttaagtctcactgaaccgttgatggagcaagtcggaacggaagagtttatcaaaaggttcggtgatggtgcttcgcgtgtagtgctcagccttcccttcgctgaggggagttctagcgttgaatatattaataactgggaacaggcgaaagcgttaagcgtagaacttgagattaattttgaaacccgtggaaaacgtggccaagatgcgatgtatgagtatatggctcaagcctgtgcaggaaatcgtgtcaggcgatctttg

SEQ ID NO: 16 - protein, 44 aa, Artificial Sequence
  Synthetic Construct
MDPDDVVDSSKSFVMENFSSYHGTKPGYVDSIQKGIQKPKSGTQ

SEQ ID NO: 17 - protein, 148 aa, Artificial Sequence
  Synthetic Construct
QGNKGFYSTDNKYDAAGYSVDNENPLSGKAGGVVKVTYPGLTKVLALKVDNAETIKKELGLSLTEPLMEQVGTEEFIKRFGDGASRVVLSLPFAEGSSSVEYINNWEQAKALSVELEINFETRGKRGQDAMYEYMAQACAGNRVRRSL

SEQ ID NO: 18 - DNA, 357 bp, Artificial Sequence
  iDTA fragment
  CDS (1)..(357)
atggatcctgatgatgttgttgattcttctaaatcttttgtgatggaaaacttttcttcgtaccacgggactaaacctggttatgtagattccattcaaaaaggtatacaaaagccaaaatctggtacacaaggaaattatgacgatgattggaaagggttttatagtaccgacaataaatacgacgctgcgggatactctgtagataatgaaaacccgctctctggaaaagctggaggcgtggtcaaagtgacgtatccaggactgacgaaggttctcgcactaaaagtggataatgccgaaactattaagaaagagttaggtttaagtctcactgaaccgttgatggagcaagtc

SEQ ID NO: 19 - protein, 119 aa, Artificial Sequence
  Synthetic Construct
MDPDDVVDSSKSFVMENFSSYHGTKPGYVDSIQKGIQKPKSGTQGNYDDDWKGFYSTDNKYDAAGYSVDNENPLSGKAGGVVKVTYPGLTKVLALKVDNAETIKKELGLSLTEPLMEQV

SEQ ID NO: 20 - DNA, 516 bp, Artificial Sequence
  NanoLuc (Nluc) gene encoding modified luciferase
  CDS (1)..(516)
atggtcttcacactcgaagatttcgttggggactggcgacagacagccggctacaacctggaccaagtccttgaacagggaggtgtgtccagtttgtttcagaatctcggggtgtccgtaactccgatccaaaggattgtcctgagcggtgaaaatgggctgaagatcgacatccatgtcatcatcccgtatgaaggtctgagcggcgaccaaatgggccagatcgaaaaaatttttaaggtggtgtaccctgtggatgatcatcactttaaggtgatcctgcactatggcacactggtaatcgacggggttacgccgaacatgatcgactatttcggacggccgtatgaaggcatcgccgtgttcgacggcaaaaagatcactgtaacagggaccctgtggaacggcaacaaaattatcgacgagcgcctgatcaaccccgacggctccctgctgttccgagtaaccatcaacggagtgaccggctggcggctgtgcgaacgcattctggcgtaa

SEQ ID NO: 21 - protein, 171 aa, Artificial Sequence
  Synthetic Construct
MVFTLEDFVGDWRQTAGYNLDQVLEQGGVSSLFQNLGVSVTPIQRIVLSGENGLKIDIHVIIPYEGLSGDQMGQIEKIFKVVYPVDDHHFKVILHYGTLVIDGVTPNMIDYFGRPYEGIAVFDGKKITVTGTLWNGNKIIDERLINPDGSLLFRVTINGVTGWRLCERILA

SEQ ID NO: 22 - DNA, 513 bp, Artificial Sequence
  SceNluc fragment
  CDS (1)..(513)
atggtcttcacactcgaagatttcgttggggactggcgacagacagccggctacaacctggaccaagtccttgaacagggaggtgtgtccagtttgtttcagaatctcggggtgtccgtaactccgatccaaaggattgtcctgagcggtgaaaatgggctgaagatcgacatccatgtcatcatcccgtatgaaggtctgagcggcgaccaaatgggccagtgatagggataacagggtaatgtgtaccctgtggatgatcatcactttaaggtgatcctgcactatggcacactggtaatcgacggggttacgccgaacatgatcgactatttcggacggccgtatgaaggcatcgccgtgttcgacggcaaaaagatcactgtaacagggaccctgtggaacggcaacaaaattatcgacgagcgcctgatcaaccccgacggctccctgctgttccgagtaaccatcaacggagtgaccggctggcggctgtgcgaacgcattctggcg

SEQ ID NO: 23 - protein, 74 aa, Artificial Sequence
  Synthetic Construct
MVFTLEDFVGDWRQTAGYNLDQVLEQGGVSSLFQNLGVSVTPIQRIVLSGENGLKIDIHVIIPYEGLSGDQMGQ

SEQ ID NO: 24 - protein, 93 aa, Artificial Sequence
  Synthetic Construct
QGNVYPVDDHHFKVILHYGTLVIDGVTPNMIDYFGRPYEGIAVFDGKKITVTGTLWNGNKIIDERLINPDGSLLFRVTINGVTGWRLCERILA

SEQ ID NO: 25 - DNA, 459 bp, Artificial Sequence
  iNluc fragment
  CDS (1)..(459)
gaagatttcgttggggactggcgacagacagccggctacaacctggaccaagtccttgaacagggaggtgtgtccagtttgtttcagaatctcggggtgtccgtaactccgatccaaaggattgtcctgagcggtgaaaatgggctgaagatcgacatccatgtcatcatcccgtatgaaggtctgagcggcgaccaaatgggccagatcgaaaaaatttttaaggtggtgtaccctgtggatgatcatcactttaaggtgatcctgcactatggcacactggtaatcgacggggttacgccgaacatgatcgactatttcggacggccgtatgaaggcatcgccgtgttcgacggcaaaaagatcactgtaacagggaccctgtggaacggcaacaaaattatcgacgagcgcctgatcaaccccgacggctccctgctgttccgagtaaccatcaac

SEQ ID NO: 26 - protein, 153 aa, Artificial Sequence
  Synthetic Construct
EDFVGDWRQTAGYNLDQVLEQGGVSSLFQNLGVSVTPIQRIVLSGENGLKIDIHVIIPYEGLSGDQMGQIEKIFKVVYPVDDHHFKVILHYGTLVIDGVTPNMIDYFGRPYEGIAVFDGKKITVTGTLWNGNKIIDERLINPDGSLLFRVTIN

SEQ ID NO: 27 - DNA, 41 bp, Artificial Sequence
  primer iNluc-Fw2
acatggctcgacagatctatgaagatttcgttggggactgg

SEQ ID NO: 28 - DNA, 45 bp, Artificial Sequence
  primer iNluc-Rv2
ggccaatattgaagatcttatcagttgatggttactcggaacagc

SEQ ID NO: 29 - DNA, 43 bp, Artificial Sequence
  primer iDTA-Fw2
acatggctcgacagatctatgacagctcttaaggctagagtac

SEQ ID NO: 30 - DNA, 39 bp, Artificial Sequence
  primer iDTA-Rv2
ggccaatattgaagatctgacttgctccatcaacggttc

SEQ ID NO: 31 - DNA, 26 bp, Artificial Sequence
  primer Sce-5'TK-Fw
cttaatacgactcactataggctagc

SEQ ID NO: 32 - DNA, 44 bp, Artificial Sequence
  primer Sce-5'TK-Rv
ttaccctgttatccctatcagatgggatggcggtcgaagatgag

SEQ ID NO: 33 - DNA, 39 bp, Artificial Sequence
  primer Sce-3'TK-Fw
gatagggataacagggtaatgccgcgcggtaccttatgg

SEQ ID NO: 34 - DNA, 20 bp, Artificial Sequence
  primer Sce-3'TK-Rv
gagtgcaccatacgcggatc

SEQ ID NO: 35 - DNA, 41 bp, Artificial Sequence
  primer iTK-Fw
acatggctcgacagatctatgcgcgtctgcgttcgaccagg

SEQ ID NO: 36 - DNA, 38 bp, Artificial Sequence
  primer iTK-Rv
ggccaatattgaagatctgtcgcatatcgtcggtatgg

SEQ ID NO: 37 - DNA, 1131 bp, herpes simplex virus
  CDS (1)..(1131)
atggcttcgtaccccggccatcaacacgcgtctgcgttcgaccaggctgcgcgttctcgcggccatagcaaccgacgtacggcgttgcgccctcgccggcagcaagaagccacggaagtccgcccggagcagaaaatgcccacgctactgcgggtttatatagacggtccccacgggatggggaaaaccaccaccacgcaactgctggtggccctgggttcgcgcgacgatatcgtctacgtacccgagccgatgacttactggcgggtgctgggggcttccgagacaatcgcgaacatctacaccacacaacaccgcctcgaccagggtgagatatcggccggggacgcggcggtggtaatgacaagcgcccagataacaatgggcatgccttatgccgtgaccgacgccgttctggctcctcatatcgggggggaggctgggagctcacatgccccgcccccggccctcaccctcatcttcgaccgccatcccatcgccgccctcctgtgctacccggccgcgcggtaccttatgggcagcatgaccccccaggccgtgctggcgttcgtggccctcatcccgccgaccttgcccggcaccaacatcgtgcttggggcccttccggaggacagacacatcgaccgcctggccaaacgccagcgccccggcgagcggctggacctggctatgctggctgcgattcgccgcgtttacgggctacttgccaatacggtgcggtatctgcagtgcggcgggtcgtggcgggaggactggggacagctttcggggacggccgtgccgccccagggtgccgagccccagagcaacgcgggcccacgaccccatatcggggacacgttatttaccctgtttcgggcccccgagttgctggcccccaacggcgacctgtataacgtgtttgcctgggccttggacgtcttggccaaacgcctccgttccatgcacgtctttatcctggattacgaccaatcgcccgccggctgccgggacgccctgctgcaacttacctccgggatggtccagacccacgtcaccacccccggctccataccgacgatatgcgacctggcgcgcacgtttgcccgggagatgggggaggctaactga

SEQ ID NO: 38 - protein, 376 aa, herpes simplex virus
MASYPGHQHASAFDQAARSRGHSNRRTALRPRRQQEATEVRPEQKMPTLLRVYIDGPHGMGKTTTTQLLVALGSRDDIVYVPEPMTYWRVLGASETIANIYTTQHRLDQGEISAGDAAVVMTSAQITMGMPYAVTDAVLAPHIGGEAGSSHAPPPALTLIFDRHPIAALLCYPAARYLMGSMTPQAVLAFVALIPPTLPGTNIVLGALPEDRHIDRLAKRQRPGERLDLAMLAAIRRVYGLLANTVRYLQCGGSWREDWGQLSGTAVPPQGAEPQSNAGPRPHIGDTLFTLFRAPELLAPNGDLYNVFAWALDVLAKRLRSMHVFILDYDQSPAGCRDALLQLTSGMVQTHVTTPGSIPTICDLARTFAREMGEAN

SEQ ID NO: 39 - DNA, 1131 bp, Artificial Sequence
  SceTK fragment
  CDS (1)..(1131)
atggcttcgtaccccggccatcaacacgcgtctgcgttcgaccaggctgcgcgttctcgcggccatagcaaccgacgtacggcgttgcgccctcgccggcagcaagaagccacggaagtccgcccggagcagaaaatgcccacgctactgcgggtttatatagacggtccccacgggatggggaaaaccaccaccacgcaactgctggtggccctgggttcgcgcgacgatatcgtctacgtacccgagccgatgacttactggcgggtgctgggggcttccgagacaatcgcgaacatctacaccacacaacaccgcctcgaccagggtgagatatcggccggggacgcggcggtggtaatgacaagcgcccagataacaatgggcatgccttatgccgtgaccgacgccgttctggctcctcatatcgggggggaggctgggagctcacatgccccgcccccggccctcaccctcatcttcgaccgccatcccatctgatagggataacagggtaatgccgcgcggtaccttatgggcagcatgaccccccaggccgtgctggcgttcgtggccctcatcccgccgaccttgcccggcaccaacatcgtgcttggggcccttccggaggacagacacatcgaccgcctggccaaacgccagcgccccggcgagcggctggacctggctatgctggctgcgattcgccgcgtttacgggctacttgccaatacggtgcggtatctgcagtgcggcgggtcgtggcgggaggactggggacagctttcggggacggccgtgccgccccagggtgccgagccccagagcaacgcgggcccacgaccccatatcggggacacgttatttaccctgtttcgggcccccgagttgctggcccccaacggcgacctgtataacgtgtttgcctgggccttggacgtcttggccaaacgcctccgttccatgcacgtctttatcctggattacgaccaatcgcccgccggctgccgggacgccctgctgcaacttacctccgggatggtccagacccacgtcaccacccccggctccataccgacgatatgcgacctggcgcgcacgtttgcccgggagatgggggaggctaactga

SEQ ID NO: 40 - protein, 166 aa, Artificial Sequence
  Synthetic Construct
MASYPGHQHASAFDQAARSRGHSNRRTALRPRRQQEATEVRPEQKMPTLLRVYIDGPHGMGKTTTTQLLVALGSRDDIVYVPEPMTYWRVLGASETIANIYTTQHRLDQGEISAGDAAVVMTSAQITMGMPYAVTDAVLAPHIGGEAGSSHAPPPALTLIFDRHPI

SEQ ID NO: 41 - protein, 206 aa, Artificial Sequence
  Synthetic Construct
QGNAARYLMGSMTPQAVLAFVALIPPTLPGTNIVLGALPEDRHIDRLAKRQRPGERLDLAMLAAIRRVYGLLANTVRYLQCGGSWREDWGQLSGTAVPPQGAEPQSNAGPRPHIGDTLFTLFRAPELLAPNGDLYNVFAWALDVLAKRLRSMHVFILDYDQSPAGCRDALLQLTSGMVQTHVTTPGSIPTICDLARTFAREMGEAN

SEQ ID NO: 42 - DNA, 1063 bp, Artificial Sequence
  iTK fragment
  CDS (2)..(1063)
cgcgtctgcgttcgaccaggctgcgcgttctcgcggccatagcaaccgacgtacggcgttgcgccctcgccggcagcaagaagccacggaagtccgcccggagcagaaaatgcccacgctactgcgggtttatatagacggtccccacgggatggggaaaaccaccaccacgcaactgctggtggccctgggttcgcgcgacgatatcgtctacgtacccgagccgatgacttactggcgggtgctgggggcttccgagacaatcgcgaacatctacaccacacaacaccgcctcgaccagggtgagatatcggccggggacgcggcggtggtaatgacaagcgcccagataacaatgggcatgccttatgccgtgaccgacgccgttctggctcctcatatcgggggggaggctgggagctcacatgccccgcccccggccctcaccctcatcttcgaccgccatcccatcgccgccctcctgtgctacccggccgcgcggtaccttatgggcagcatgaccccccaggccgtgctggcgttcgtggccctcatcccgccgaccttgcccggcaccaacatcgtgcttggggcccttccggaggacagacacatcgaccgcctggccaaacgccagcgccccggcgagcggctggacctggctatgctggctgcgattcgccgcgtttacgggctacttgccaatacggtgcggtatctgcagtgcggcgggtcgtggcgggaggactggggacagctttcggggacggccgtgccgccccagggtgccgagccccagagcaacgcgggcccacgaccccatatcggggacacgttatttaccctgtttcgggcccccgagttgctggcccccaacggcgacctgtataacgtgtttgcctgggccttggacgtcttggccaaacgcctccgttccatgcacgtctttatcctggattacgaccaatcgcccgccggctgccgggacgccctgctgcaacttacctccgggatggtccagacccacgtcaccacccccggctccataccgacgatatgcgac

SEQ ID NO: 43 - protein, 354 aa, Artificial Sequence
  Synthetic Construct
ASAFDQAARSRGHSNRRTALRPRRQQEATEVRPEQKMPTLLRVYIDGPHGMGKTTTTQLLVALGSRDDIVYVPEPMTYWRVLGASETIANIYTTQHRLDQGEISAGDAAVVMTSAQITMGMPYAVTDAVLAPHIGGEAGSSHAPPPALTLIFDRHPIAALLCYPAARYLMGSMTPQAVLAFVALIPPTLPGTNIVLGALPEDRHIDRLAKRQRPGERLDLAMLAAIRRVYGLLANTVRYLQCGGSWREDWGQLSGTAVPPQGAEPQSNAGPRPHIGDTLFTLFRAPELLAPNGDLYNVFAWALDVLAKRLRSMHVFILDYDQSPAGCRDALLQLTSGMVQTHVTTPGSIPTICD

SEQ ID NO: 44 - DNA, 600 bp, Artificial Sequence
  SecNluc gene
  CDS (1)..(600)
atgaactccttctccacaagcgccttcggtccagttgccttctccctgggcctgctcctggtgttgcctgctgccttccctgccccagtcttcacactcgaagatttcgttggggactggcgacagacagccggctacaacctggaccaagtccttgaacagggaggtgtgtccagtttgtttcagaatctcggggtgtccgtaactccgatccaaaggattgtcctgagcggtgaaaatgggctgaagatcgacatccatgtcatcatcccgtatgaaggtctgagcggcgaccaaatgggccagatcgaaaaaatttttaaggtggtgtaccctgtggatgatcatcactttaaggtgatcctgcactatggcacactggtaatcgacggggttacgccgaacatgatcgactatttcggacggccgtatgaaggcatcgccgtgttcgacggcaaaaagatcactgtaacagggaccctgtggaacggcaacaaaattatcgacgagcgcctgatcaaccccgacggctccctgctgttccgagtaaccatcaacggagtgaccggctggcggctgtgcgaacgcattctggcgtaa

SEQ ID NO: 45 - protein, 199 aa, Artificial Sequence
  Synthetic Construct
MNSFSTSAFGPVAFSLGLLLVLPAAFPAPVFTLEDFVGDWRQTAGYNLDQVLEQGGVSSLFQNLGVSVTPIQRIVLSGENGLKIDIHVIIPYEGLSGDQMGQIEKIFKVVYPVDDHHFKVILHYGTLVIDGVTPNMIDYFGRPYEGIAVFDGKKITVTGTLWNGNKIIDERLINPDGSLLFRVTINGVTGWRLCERILA

SEQ ID NO: 46 - DNA, 600 bp, Artificial Sequence
  SceSecNluc gene
  CDS (1)..(600)
atgaactccttctccacaagcgccttcggtccagttgccttctccctgggcctgctcctggtgttgcctgctgccttccctgccccagtcttcacactcgaagatttcgttggggactggcgacagacagccggctacaacctggaccaagtccttgaacagggaggtgtgtccagtttgtttcagaatctcggggtgtccgtaactccgatccaaaggattgtcctgagcggtgaaaatgggctgaagatcgacatccatgtcatcatcccgtatgaaggtctgagcggcgaccaaatgggccagtgatagggataacagggtaatgtgtaccctgtggatgatcatcactttaaggtgatcctgcactatggcacactggtaatcgacggggttacgccgaacatgatcgactatttcggacggccgtatgaaggcatcgccgtgttcgacggcaaaaagatcactgtaacagggaccctgtggaacggcaacaaaattatcgacgagcgcctgatcaaccccgacggctccctgctgttccgagtaaccatcaacggagtgaccggctggcggctgtgcgaacgcattctggcgtaa

SEQ ID NO: 47 - protein, 102 aa, Artificial Sequence
  Synthetic Construct
MNSFSTSAFGPVAFSLGLLLVLPAAFPAPVFTLEDFVGDWRQTAGYNLDQVLEQGGVSSLFQNLGVSVTPIQRIVLSGENGLKIDIHVIIPYEGLSGDQMGQ

SEQ ID NO: 48 - protein, 93 aa, Artificial Sequence; identical to SEQ ID NO: 24
  Synthetic Construct